European Patent Application EP 4 553 165 A1, published May 14, 2025. Title: METHOD FOR DETECTING FUSOBACTERIUM NUCLEATUM AND METHOD FOR DETECTING FUSOBACTERIUM NUCLEATUM SUBSP. NUCLEATUM. Applicant: 栄研化学株式会社. Application JP. The sequence listing filed with the application follows.

SEQUENCE LISTING (73 sequences)

SEQ ID NO: 1 - DNA, 891 bp, Fusobacterium nucleatum subsp. nucleatum
  source 1..891: mol_type = genomic DNA
  CDS 1..891: protein_id = 69; translation = MAIRDRLRRTMMFLPGNNPSMITDAYIYGPDSVMIDLEDATSVNQKDAARFLVSEALKTIDYKTTETVVRVNGLDTPFGADDIRAVVKAGVNVVRLPKTDTPNEIIAVDKLITEVEKEIGREGETLLMAAIESATGIMNVKEIALASKRLMGIALGAEDYVTNLKTSRSKHGWELYYAREAIVLAARNAGIYCFDTVYSDVNNLDGFRQEVQFIKDLGFDGKSCIHPKQVRIVHEIYTPTQKEIEKSIRIINGAKEAEAKGSGVISVDGKMVDNPIIMRAQRVLELAKASGIYKED
atggcaattagagatagattaagaagaactatgatgtttctacctggtaataatccatcaatgattacagatgcttatatatatggaccagattctgtaatgattgacttagaagatgctactagtgtaaatcaaaaagatgctgcgagatttttagtttctgaagctttaaaaacaatagattataaaactactgaaactgttgtaagagtaaatggtttagacactccatttggggcagatgacataagagctgttgttaaagctggagtaaatgttgtaagacttccaaaaacagatactcctaatgaaataatagctgttgataaattaataacagaagttgaaaaagaaataggtagagagggagaaactctacttatggcagctattgaaagtgcaactggtattatgaatgttaaagaaattgctcttgctagtaaaagattaatgggaattgcattaggagcagaagattatgttactaacttaaagacttcaagaagtaaacatggttgggaactatactatgcaagagaagctattgtacttgctgcaagaaatgctggtatttattgctttgatactgtttattcagatgtaaataacttagatggtttcagacaagaagtgcaatttattaaagatttgggatttgatggaaaatcttgtatacaccctaaacaagttagaatagttcatgaaatttatacaccgactcaaaaagaaattgaaaagtcaattagaattataaatggtgctaaagaagctgaagctaagggttcaggagttatatctgttgatggtaaaatggttgataacccaattattatgagagctcaaagagtactagaattagcaaaagctagtgggatttacaaggaggactaa

SEQ ID NO: 2 - DNA, 891 bp, Fusobacterium nucleatum subsp. animalis
  source 1..891: mol_type = genomic DNA
  CDS 1..891: protein_id = 70; translation = MAIRDRLRRTMMFLPGNNPSMITDAYIYGPDSVMIDLEDATSVNQKDAARFLVSEALKTIDYKTTETVVRVNGLDTPFGADDIRAVVKAGVNVVRLPKTDTPDEIIAVDKLITEVEKEIGREGETLLMAAIESATGIMNVKEIALASKRLMGIALGAEDYVTNLKTSRSKHGWELYYAREAIVLAARNAGIYCFDTVYSDVNNLDGFRQEVQFIKDLGFDGKSCIHPKQVRIVHEIYTPSQKEIEKSIRIINGAKEAEAKGSGVISVDGKMVDNPIIMRAQRVLELAKASGIYKED
atggcaattagagatagattaagaagaacaatgatgtttctacctggtaataatccatcaatgattacagatgcttatatatatggaccagattctgtaatgatagacttagaagatgctactagtgtaaatcaaaaagatgctgcaagatttttagtttctgaggctttaaaaacaatagattataaaactactgaaactgttgtaagggtaaatggtttagatactccatttggagcagatgatataagagctgttgtaaaagcaggagttaatgttgtaagacttccaaaaactgatactcctgatgaaataatagcagttgataaacttataacagaagttgaaaaagaaattggtagagaaggagaaactctacttatggcagctattgaaagtgcaactggtattatgaatgttaaagaaattgctcttgctagcaaaagattaatgggtatagcattaggagcagaagactatgttactaacttaaagacttcaagaagtaaacatggttgggaattatattatgcaagagaagctattgtgcttgctgcaagaaatgcgggtatttattgctttgatactgtttattcagatgtaaataacctagatggtttcagacaagaagttcaatttattaaagatttaggatttgatggtaaatcttgtatacatcctaaacaagttagaatagttcatgaaatttatacaccaagccaaaaagaaattgaaaaatcaatcagaattataaatggtgctaaggaagctgaagctaagggttcaggagttatatctgttgatggtaaaatggttgataacccaattattatgagagctcaaagagttttagaattagcaaaagctagtggtatttataaggaggactaa

SEQ ID NO: 3 - DNA, 891 bp, Fusobacterium nucleatum subsp. polymorphum
  source 1..891: mol_type = genomic DNA
  CDS 1..891: protein_id = 71; translation = MAIRDRLRRTMMFLPGNNPSMITDAYIYGPDSVMIDLEDATSVNQKDAARFLVSEALKTIDYKTTETVVRVNGLDTPFGADDIRAVVKAGVNVVRLPKTDTPDEIIAVDKLITEVEKEIGREGETLLMAAIESATGIMNVKEIALASKRLMGIALGAEDYVTNLKTSRSKHGWELYYAREAIVLAARNAGIYCFDTVYSDVNNLDGFRQEVQFIKDLGFDGKSCIHPKQVRIVHEIYTPTQKEIEKSIRIINGAKEAEAKGSGVISVDGKMVDNPIIMRAQRVLELAKASGIYKED
atggcaattagagatagattaagaagaactatgatgtttttacctggtaataatccatcaatgattacagatgcctatatatatggaccagattctgtaatgatagacttggaagatgctactagtgtaaaccaaaaagatgctgcaagatttttagtttctgaagctttaaaaacaatagactataaaactaccgaaactgttgtaagggtaaatggtttagatactccatttggagcagatgatataagagctgttgttaaagcaggagttaatgttgtaagacttccaaaaactgatactcctgatgaaataatagcagttgataaacttataacagaagttgaaaaagaaattggtagagaaggagaaactctacttatggcagctattgaaagtgcaactggtattatgaatgttaaagaaattgctcttgctagcaaaagattaatgggtatagcattaggagcagaagactatgttactaacttaaagacttcaagaagtaaacatggttgggaattatattatgcaagagaagctattgtgcttgctgcaagaaatgcgggtatttattgctttgatactgtttattcagatgtaaataacctagatggtttcagacaagaagttcaatttattaaagatttaggatttgatggaaaatcttgtatacatcctaaacaagttagaatagttcatgaaatttatacaccaactcaaaaagaaattgaaaaatcaattagaattataaatggtgctaaagaagctgaagctaagggttcaggagttatatctgttgatggtaaaatggttgataacccaattattatgagagctcaaagagttttagaattagcaaaagctagtgggatttataaggaggactaa

SEQ ID NO: 4 - DNA, 891 bp, Fusobacterium nucleatum subsp. vincentii
  source 1..891: mol_type = genomic DNA
  CDS 1..891: protein_id = 72; translation = MAIRDRLRRTMMFLPGNNPSMITDAYIYGPDSVMIDLEDATSVNQKDAARFLVSEALKTIDYKTTETVVRVNGLDTPFGADDIRAVVKAGVNVVRLPKTDTPDEIIAVDKLITEVEKEIGREGETLLMAAIESATGIMNVKEIALASKRLMGIALGAEDYVTNLKTSRSKHGWELYYAREAIVLAARNAGIYCFDTVYSDVNNLDGFRQEVQFIKDLGFDGKSCIHPKQVRIVHEIYTPSQKEIEKSIRIINGAKEAEAKGSGVISVDGKMVDNPIIMRAQRVLELAKASGIYKED
atggcaattagagatagattaagaagaacaatgatgtttctacctggtaataatccatcaatgattacagatgcttatatatatggaccagattctgtaatgatagacttagaagatgctaccagtgtaaatcaaaaagatgctgcaagatttttagtttctgaggctttaaaaacaatagattataaaactactgaaactgttgtaagagtaaatggtttagatactccatttggagctgatgatataagagctgttgttaaagcaggagttaatgttgtaagacttccaaaaacagatactcctgatgaaataatagcagttgataaacttataacagaagttgaaaaagaaattggtagagaaggagaaactctacttatggcagctattgaaagtgcaactggtattatgaatgttaaagaaattgctcttgctagcaaaagattaatgggaatagcattaggagcagaagactatgttactaacttaaagacttcaagaagtaaacatggttgggaattatattatgcaagagaagctattgtacttgctgcaagaaatgcaggtatttattgttttgatactgtttattcagatgtaaataacctagatggtttcagacaagaagttcaatttattaaagatttaggatttgatggtaaatcttgtatacaccctaaacaagttagaatagttcatgaaatttatacaccaagccaaaaagaaattgaaaaatcaattagaattataaatggtgctaaggaagctgaagctaagggttcaggagttatatcagttgatggtaaaatggttgataacccaattattatgagagctcaaagagttttagaattagcaaaagctagtggaatttataaggaggactaa

SEQ ID NO: 5 - DNA, 23 bp, synthetic construct
  source 1..23: mol_type = other DNA
tgctgcaagatttttagtttctg

SEQ ID NO: 6 - DNA, 22 bp, synthetic construct
  source 1..22: mol_type = other DNA
tcataataccagttgcactttc

SEQ ID NO: 7 - DNA, 52 bp, synthetic construct
  source 1..52: mol_type = other DNA
ttggaagtcttacaacattaacccctagactataaaactactgaaactgttg

SEQ ID NO: 8 - DNA, 45 bp, synthetic construct
  source 1..45: mol_type = other DNA
actcctgatgaaataatagcagttggccataagtagagtttctcc

SEQ ID NO: 9 - DNA, 28 bp, synthetic construct
  source 1..28: mol_type = other DNA
ctcttatatcatctgctccaaatggagt

SEQ ID NO: 10 - DNA, 31 bp, synthetic construct
  source 1..31: mol_type = other DNA
aacagaagttgaaaaagaaattggtagagaa

SEQ ID NO: 11 - DNA, 1209 bp, Fusobacterium nucleatum subsp. nucleatum
  source 1..1209: mol_type = genomic DNA
  CDS 1..1209: protein_id = 73; translation = MKKLALWKQIIIAILLGILVGVFMPNIVPKFKFLGDIFLRLLKMLIAPLVLFTLISGVCKMGDIKQLRTVGMRIVIFYLASSTVSAILGVLIALFTQPGKGVIDLLGTEVGKDVSYNFIENLIGWVPINIFEALATGNTLQIIFFALLMGVVLLSLGDSVSVVIKIVDQAADAMMKLTEIVMKFAPIGIFALIADLTISLSGNMLKQVLNMILTVYIVLLFIIFIVYPIAIKLFTKESGLKFLKNVTPAMIVAASTTSSAATLPVSLRCANEELGVPENIFGFTLPLGNTCNMNGLAVGLGVISVFASNIYGYPITFVSLLQFVFMGLVLSVGCAGVKGAGIVMSTVLLQTFGMPLTLIPILAAIWPITDIGYTTANITGDLVGTVVVANSLNSLDKEIFRK
atgaaaaaattagcattatggaaacaaataataatagctattctattaggaattttagtaggagtttttatgcctaatattgtaccaaaatttaaatttttgggagatatatttttaagacttttaaaaatgctaatagcaccacttgttttgttcactttaataagtggtgtatgtaaaatgggggatatcaaacaattaagaacagttggaatgagaatagttattttctatcttgcttcctcaactgtttcagcaatattaggagttttaattgctttgtttactcaaccaggaaagggagttatagatttattaggtactgaagttggaaaagatgttagttataatttcattgaaaatttaattggctgggtccctataaatatatttgaagcattagcaacaggaaatacattacagattatcttttttgctctattaatgggagttgttttattgagcttgggagattctgtaagtgtggttataaaaattgtagatcaagcagcagatgctatgatgaaattaacagaaattgttatgaaatttgcacccattgggatttttgcgttaatagctgatttaactatttctttatctggaaatatgttaaaacaagtattaaacatgatactaactgtctacatagttttattgttcataatatttatagtttatcctatagcaataaaattattcacaaaggaaagtggactgaaatttttgaaaaatgttactcctgcaatgattgtagctgcctcaacaacatcttctgcagcaactttaccagtttctttaagatgtgcaaatgaagaattaggagttcctgaaaatatatttggttttactttaccattaggaaatacttgtaatatgaatggtttagctgttggattaggtgtaataagtgtatttgcttcaaatatttatggttatccaataacttttgtatcattacttcaatttgtatttatgggattagttctttcggttggatgtgctggggtaaaaggtgcaggaatagttatgtcaacagttttattacaaacatttggaatgcctttaacactgataccaattttagcagctatatggcctataactgatatcggatatactactgccaatataacaggagatttagtaggcactgttgttgttgctaattcattaaatagtttagataaggaaatttttagaaaataa

SEQ ID NO: 12 - DNA, 26 bp, synthetic construct
  source 1..26: mol_type = other DNA
taggaaatacttgtaatatgaatggt

SEQ ID NO: 13 - DNA, 24 bp, synthetic construct
  source 1..24: mol_type = other DNA
gtatatccgatatcagttataggc

SEQ ID NO: 14 - DNA, 53 bp, synthetic construct
  source 1..53: mol_type = other DNA
cgaaagaactaatcccataaatacaaattggttggattaggtgtaataagtgt

SEQ ID NO: 15 - DNA, 43 bp, synthetic construct
  source 1..43: mol_type = other DNA
ggatgtgctggggtaaaaggagctgctaaaattggtatcagtg

SEQ ID NO: 16 - DNA, 44 bp, synthetic construct
  source 1..44: mol_type = other DNA
agtaatgatacaaaagttattggataaccataaatatttgaagc

SEQ ID NO: 17 - DNA, 33 bp, synthetic construct
  source 1..33: mol_type = other DNA
gtcaacagttttattacaaacatttggaatgcc

SEQ ID NO: 18 - DNA, 1000 bp, synthetic construct
  source 1..1000: mol_type = other DNA
ctataaaagaattaggtgttgaaaatgctaatgtaaaagttgtagataagggtgcattaaactatgctcttatagctagaactaaagctgctgtatatagagctgctgaatctaatgattataaattttaggaggaattatggcaattagagatagattaagaagaacaatgatgtttctacctggaaacaatccgtcaatgattacagatgctcatatttataaaccagactctataatgattgacttagaggatgctgtaagtgtaaatcaaaaagatgctgctagatttttagtttctgaagcattaaaagcaatagattacaaaacaactgaaagagttgtaagagtaaatggtttggatactccatttggagcagatgatataagagcgattgtaaaagctggagttgatgtaataagacttcctaagactgacaaccctgacgaaataattgctgttgataaattaataacagaagttgaaaaagaaattggtagagaaggagaaactctacttatggcagctattgaaagtgcagctggtattatgaatgttaaagaaattgctcttgctagtaaaagattaatgggaatagctctaggagcagaagactatgttactaacttaaaaacttcaagaagtaaacatggttgggaactatactatgcaagggaagctattgtacttgctgcaagaaatgctggtatttattgttttgatactgtttactcagatgtaaataacttagaaggttttagaaatgaagttcaattcattaaagatttaggatttgatggaaaatcttgtatacatcctaaacaagttagaatagttcatgaaatttatacaccaactcaaaaagaaattgaaaaatcaattagaattataaatggtgccaaagaggcagaagctaagggttcaggagttatatctgttgatggtaaaatggttgataacccaattattatgagagctcaaagagtgctagaattagca

SEQ ID NO: 19 - DNA, 23 bp, synthetic construct
  source 1..23: mol_type = other DNA
aatactacgattcattgacaaga

SEQ ID NO: 20 - DNA, 24 bp, synthetic construct
  source 1..24: mol_type = other DNA
gttaattcctcaagaataccgata

SEQ ID NO: 21 - DNA, 61 bp, synthetic construct
  source 1..61: mol_type = other DNA
gtttgtgctgtaattataacacctttttaaagttagagaaaataatgatatgatttcatgg

SEQ ID NO: 22 - DNA, 59 bp, synthetic construct
  source 1..59: mol_type = other DNA
tgactgtaaaaaattatgaagaaaaagtttctcgctttaatatattattaactgttgga

SEQ ID NO: 23 - DNA, 27 bp, synthetic construct
  source 1..27: mol_type = other DNA
agagaaaataatgatatgatttcatgg

SEQ ID NO: 24 - DNA, 30 bp, synthetic construct
  source 1..30: mol_type = other DNA
ccttctataaatattgaaagatattccatt

SEQ ID NO: 25 - DNA, 55 bp, synthetic construct
  source 1..55: mol_type = other DNA
agaaactttttcttcataattttttacagtcaaaaggtgttataattacagcaca

SEQ ID NO: 26 - DNA, 59 bp, synthetic construct
  source 1..59: mol_type = other DNA
gttttccaacagttaataatatattaaagcgttcttttataattggttaattcctcaag

SEQ ID NO: 27 - DNA, 20 bp, synthetic construct
  source 1..20: mol_type = other DNA
gggagattgatgatacctct

SEQ ID NO: 28 - DNA, 28 bp, synthetic construct
  source 1..28: mol_type = other DNA
ctttttcttcataattttttacagtcat

SEQ ID NO: 29 - DNA, 63 bp, synthetic construct
  source 1..63: mol_type = other DNA
gaatcgtagtattctgttctatttttttcaaattgctagataaaatatattgaataaaccatg

SEQ ID NO: 30 - DNA, 51 bp, synthetic construct
  source 1..51: mol_type = other DNA
attgacaagagttagagaaaataatgatatgatcttagctgtttgtgctgt

SEQ ID NO: 31 - DNA, 26 bp, synthetic construct
  source 1..26: mol_type = other DNA
gcaattagagatagattaagaagaac

SEQ ID NO: 32 - DNA, 23 bp, synthetic construct
  source 1..23: mol_type = other DNA
ctcttatatcatctgctccaaat

SEQ ID NO: 33 - DNA, 50 bp, synthetic construct
  source 1..50: mol_type = other DNA
tttacactagtagcatcttctaagtcctacctggtaataatccatcaatg

SEQ ID NO: 34 - DNA, 55 bp, synthetic construct
  source 1..55: mol_type = other DNA
caaaaagatgctgcaagatttttagtttctgctaaaccatttacycttacaacag

SEQ ID NO: 35 - DNA, 30 bp, synthetic construct
  source 1..30: mol_type = other DNA
atctggtccatatatataagcatctgtaat

SEQ ID NO: 36 - DNA, 34 bp, synthetic construct
  source 1..34: mol_type = other DNA
gctttaaaaacaatagattataaaactactgaaa

SEQ ID NO: 37 - DNA, 22 bp, synthetic construct
  source 1..22: mol_type = other DNA
gcagatgatataagagctgttg

SEQ ID NO: 38 - DNA, 18 bp, synthetic construct
  source 1..18: mol_type = other DNA
tcttgcagcaagcacaat

SEQ ID NO: 39 - DNA, 54 bp, synthetic construct
  source 1..54: mol_type = other DNA
ccattaatcttttgctagcaagagcaagagttaatgttgtaagacttccaaaaa

SEQ ID NO: 40 - DNA, 49 bp, synthetic construct
  source 1..49: mol_type = other DNA
aggagcagaagactatgttactaactcttgcataatataattcccaacc

SEQ ID NO: 41 - DNA, 30 bp, synthetic construct
  source 1..30: mol_type = other DNA
tttctttaacattcataataccagttgcac

SEQ ID NO: 42 - DNA, 28 bp, synthetic construct
  source 1..28: mol_type = other DNA
taacttaaagacttcaagaagtaaacat

SEQ ID NO: 43 - DNA, 23 bp, synthetic construct
  source 1..23: mol_type = other DNA
tgctttgatactgtttattcaga

SEQ ID NO: 44 - DNA, 23 bp, synthetic construct
  source 1..23: mol_type = other DNA
ccatcaacagatataactcctga

SEQ ID NO: 45 - DNA, 51 bp, synthetic construct
  source 1..51: mol_type = other DNA
tgtatacaagatttaccatcaaatccgtaaataacctagatggtttcagac

SEQ ID NO: 46 - DNA, 48 bp, synthetic construct
  source 1..48: mol_type = other DNA
ttagaatagttcatgaaatttatacaccaaacccttagcttcagcttc

SEQ ID NO: 47 - DNA, 33 bp, synthetic construct
  source 1..33: mol_type = other DNA
caaatcctaaatctttaataaattgaacttctt

SEQ ID NO: 48 - DNA, 35 bp, synthetic construct
  source 1..35: mol_type = other DNA
aaaaagaaattgaaaaatcaatcagaattataaat

SEQ ID NO: 49 - DNA, 25 bp, synthetic construct
  source 1..25: mol_type = other DNA
caattaagaacagttggaatgagaa

SEQ ID NO: 50 - DNA, 30 bp, synthetic construct
  source 1..30: mol_type = other DNA
cccattaatagagcaaaaaagataatctgt

SEQ ID NO: 51 - DNA, 48 bp, synthetic construct
  source 1..48: mol_type = other DNA
taactccctttcctggttgagtatctatcttgcttcctcaactgtttc

SEQ ID NO: 52 - DNA, 47 bp, synthetic construct
  source 1..47: mol_type = other DNA
taggtactgaagttggaaaagatgtttgtatttcctgttgctaatgc

SEQ ID NO: 53 - DNA, 29 bp, synthetic construct
  source 1..29: mol_type = other DNA
aacaaagcaattaaaactcctaatattgc

SEQ ID NO: 54 - DNA, 26 bp, synthetic construct
  source 1..26: mol_type = other DNA
attgaaaatttaattggctgggtccc

SEQ ID NO: 55 - DNA, 26 bp, synthetic construct
  source 1..26: mol_type = other DNA
gctgatttaactatttctttatctgg

SEQ ID NO: 56 - DNA, 26 bp, synthetic construct
  source 1..26: mol_type = other DNA
gtatttcctaatggtaaagtaaaacc

SEQ ID NO: 57 - DNA, 60 bp, synthetic construct
  source 1..60: mol_type = other DNA
tccactttcctttgtgaataattttattgccaagtattaaacatgatactaactgtctac

SEQ ID NO: 58 - DNA, 47 bp, synthetic construct
  source 1..47: mol_type = other DNA
tgttactcctgcaatgattgtagctttcaggaactcctaattcttca

SEQ ID NO: 59 - DNA, 36 bp, synthetic construct
  source 1..36: mol_type = other DNA
aggataaactataaatattatgaacaataaaactat

SEQ ID NO: 60 - DNA, 23 bp, synthetic construct
  source 1..23: mol_type = other DNA
catcttctgcagcaactttacca

SEQ ID NO: 61 - DNA, 20 bp, synthetic construct
  source 1..20: mol_type = other DNA
cctcaacaacatcttctgca

SEQ ID NO: 62 - DNA, 22 bp, synthetic construct
  source 1..22: mol_type = other DNA
tgttgacataactattcctgca

SEQ ID NO: 63 - DNA, 56 bp, synthetic construct
  source 1..56: mol_type = other DNA
ccattcatattacaagtatttcctaatggtctttaccagtttctttaagatgtgca

SEQ ID NO: 64 - DNA, 50 bp, synthetic construct
  source 1..50: mol_type = other DNA
tggattaggtgtaataagtgtatttgctaaccgaaagaactaatcccata

SEQ ID NO: 65 - DNA, 32 bp, synthetic construct
  source 1..32: mol_type = other DNA
aaagtaaaaccaaatatattttcaggaactcc

SEQ ID NO: 66 - DNA, 34 bp, synthetic construct
  source 1..34: mol_type = other DNA
atggttatccaataacttttgtatcattacttca

SEQ ID NO: 67 - DNA, 28 bp, synthetic construct
  source 1..28: mol_type = other DNA
tgatgtttctacctggtaataatccatc

SEQ ID NO: 68 - DNA, 24 bp, synthetic construct
  source 1..24: mol_type = other DNA
ttgaacttcttgtctgaaaccatc

SEQ ID NO: 69 - protein, 296 aa, Fusobacterium nucleatum subsp. nucleatum
MAIRDRLRRTMMFLPGNNPSMITDAYIYGPDSVMIDLEDATSVNQKDAARFLVSEALKTIDYKTTETVVRVNGLDTPFGADDIRAVVKAGVNVVRLPKTDTPNEIIAVDKLITEVEKEIGREGETLLMAAIESATGIMNVKEIALASKRLMGIALGAEDYVTNLKTSRSKHGWELYYAREAIVLAARNAGIYCFDTVYSDVNNLDGFRQEVQFIKDLGFDGKSCIHPKQVRIVHEIYTPTQKEIEKSIRIINGAKEAEAKGSGVISVDGKMVDNPIIMRAQRVLELAKASGIYKED

SEQ ID NO: 70 - protein, 296 aa, Fusobacterium nucleatum subsp. animalis
MAIRDRLRRTMMFLPGNNPSMITDAYIYGPDSVMIDLEDATSVNQKDAARFLVSEALKTIDYKTTETVVRVNGLDTPFGADDIRAVVKAGVNVVRLPKTDTPDEIIAVDKLITEVEKEIGREGETLLMAAIESATGIMNVKEIALASKRLMGIALGAEDYVTNLKTSRSKHGWELYYAREAIVLAARNAGIYCFDTVYSDVNNLDGFRQEVQFIKDLGFDGKSCIHPKQVRIVHEIYTPSQKEIEKSIRIINGAKEAEAKGSGVISVDGKMVDNPIIMRAQRVLELAKASGIYKED

SEQ ID NO: 71 - protein, 296 aa, Fusobacterium nucleatum subsp. polymorphum
MAIRDRLRRTMMFLPGNNPSMITDAYIYGPDSVMIDLEDATSVNQKDAARFLVSEALKTIDYKTTETVVRVNGLDTPFGADDIRAVVKAGVNVVRLPKTDTPDEIIAVDKLITEVEKEIGREGETLLMAAIESATGIMNVKEIALASKRLMGIALGAEDYVTNLKTSRSKHGWELYYAREAIVLAARNAGIYCFDTVYSDVNNLDGFRQEVQFIKDLGFDGKSCIHPKQVRIVHEIYTPTQKEIEKSIRIINGAKEAEAKGSGVISVDGKMVDNPIIMRAQRVLELAKASGIYKED

SEQ ID NO: 72 - protein, 296 aa, Fusobacterium nucleatum subsp. vincentii; identical to SEQ ID NO: 70

SEQ ID NO: 73 - protein, 402 aa, Fusobacterium nucleatum subsp. nucleatum
MKKLALWKQIIIAILLGILVGVFMPNIVPKFKFLGDIFLRLLKMLIAPLVLFTLISGVCKMGDIKQLRTVGMRIVIFYLASSTVSAILGVLIALFTQPGKGVIDLLGTEVGKDVSYNFIENLIGWVPINIFEALATGNTLQIIFFALLMGVVLLSLGDSVSVVIKIVDQAADAMMKLTEIVMKFAPIGIFALIADLTISLSGNMLKQVLNMILTVYIVLLFIIFIVYPIAIKLFTKESGLKFLKNVTPAMIVAASTTSSAATLPVSLRCANEELGVPENIFGFTLPLGNTCNMNGLAVGLGVISVFASNIYGYPITFVSLLQFVFMGLVLSVGCAGVKGAGIVMSTVLLQTFGMPLTLIPILAAIWPITDIGYTTANITGDLVGTVVVANSLNSLDKEIFRK